European Patent Application EP 4 155 418 A1, published March 29, 2023. Title: Single Nucleic Acid for Real-Time Detection for SNP Analysis of ApoE Gene and Detection Method Using the Same. Applicant: NuriBio Co., Ltd. Application EP. The sequence listing filed with the application follows.

SEQUENCE LISTING (104 sequences)

SEQ ID NO: 1 - DNA, 21 bp, Artificial Sequence
  ApoE_F primer
gaaggcctacaaatcggaact

SEQ ID NO: 2 - DNA, 17 bp, Artificial Sequence
  ApoE_R primer
gccacctgctccttcac

SEQ ID NO: 3 - DNA, 16 bp, Artificial Sequence
  Single nucleic acid type 1 for detecting SNP in 112 codon of ApoE gene
  RNA is located at 10th of sequence.
gaggacgtgugcggcc

SEQ ID NO: 4 - DNA, 16 bp, Artificial Sequence
  Single nucleic acid type 1 for detecting SNP in 112 codon of ApoE gene
  RNA is located at 10th of sequence.
gaggacgtgcgcggcc

SEQ ID NO: 5 - DNA, 18 bp, Artificial Sequence
  Single nucleic acid type 1 for detecting SNP in 152 codon of ApoE gene
  RNA is located at 10th of sequence.
ctgcagaagugcctggca

SEQ ID NO: 6 - DNA, 16 bp, Artificial Sequence
  Single nucleic acid type 1 for detecting SNP in 152 codon of ApoE gene
  RNA is located at 8th of sequence.
gcagaagcgcctggca

SEQ ID NO: 7 - DNA, 20 bp, Artificial Sequence
  Single nucleic acid type 2 for detecting SNP in 112 codon of ApoE gene
  RNA is located at 18th of sequence.
cggtcatggaggacgtgugc

SEQ ID NO: 8 - DNA, 20 bp, Artificial Sequence
  Single nucleic acid type 2 for detecting SNP in 112 codon of ApoE gene
  RNA is located at 18th of sequence.
gcggatatggaggacgtgcg

SEQ ID NO: 9 - DNA, 21 bp, Artificial Sequence
  Single nucleic acid type 2 for detecting SNP in 152 codon of ApoE gene
  RNA is located at 19th of sequence.
ctggtacactgccaggcactt

SEQ ID NO: 10 - DNA, 22 bp, Artificial Sequence
  Single nucleic acid type 2 for detecting SNP in 152 codon of ApoE gene
  RNA is located at 18th of sequence.
ctggtacactgccaggcgattc

SEQ ID NO: 11 - DNA, 4 bp, Artificial Sequence
  X part of Single nucleic acid for detecting SNP in 112 codon of ApoE gene
cgtg

SEQ ID NO: 12 - DNA, 5 bp, Artificial Sequence
  X part of Single nucleic acid for detecting SNP in 112 codon of ApoE gene
acgtg

SEQ ID NO: 13 - DNA, 6 bp, Artificial Sequence
  X part of Single nucleic acid for detecting SNP in 112 codon of ApoE gene
gacgtg

SEQ ID NO: 14 - DNA, 7 bp, Artificial Sequence
  X part of Single nucleic acid for detecting SNP in 112 codon of ApoE gene
ggacgtg

SEQ ID NO: 15 - DNA, 8 bp, Artificial Sequence
  X part of Single nucleic acid for detecting SNP in 112 codon of ApoE gene
aggacgtg

SEQ ID NO: 16 - DNA, 9 bp, Artificial Sequence
  X part of Single nucleic acid for detecting SNP in 112 codon of ApoE gene
gaggacgtg

SEQ ID NO: 17 - DNA, 10 bp, Artificial Sequence
  X part of Single nucleic acid for detecting SNP in 112 codon of ApoE gene
ggaggacgtg

SEQ ID NO: 18 - DNA, 11 bp, Artificial Sequence
  X part of Single nucleic acid for detecting SNP in 112 codon of ApoE gene
tggaggacgtg

SEQ ID NO: 19 - DNA, 12 bp, Artificial Sequence
  X part of Single nucleic acid for detecting SNP in 112 codon of ApoE gene
atggaggacgtg

SEQ ID NO: 20 - DNA, 13 bp, Artificial Sequence
  X part of Single nucleic acid for detecting SNP in 112 codon of ApoE gene
catggaggacgtg

SEQ ID NO: 21 - DNA, 14 bp, Artificial Sequence
  X part of Single nucleic acid for detecting SNP in 112 codon of ApoE gene
acatggaggacgtg

SEQ ID NO: 22 - DNA, 15 bp, Artificial Sequence
  X part of Single nucleic acid for detecting SNP in 112 codon of ApoE gene
gacatggaggacgtg

SEQ ID NO: 23 - DNA, 16 bp, Artificial Sequence
  X part of Single nucleic acid for detecting SNP in 112 codon of ApoE gene
ggacatggaggacgtg

SEQ ID NO: 24 - DNA, 17 bp, Artificial Sequence
  X part of Single nucleic acid for detecting SNP in 112 codon of ApoE gene
cggacatggaggacgtg

SEQ ID NO: 25 - DNA, 18 bp, Artificial Sequence
  X part of Single nucleic acid for detecting SNP in 112 codon of ApoE gene
gcggacatggaggacgtg

SEQ ID NO: 26 - DNA, 19 bp, Artificial Sequence
  X part of Single nucleic acid for detecting SNP in 112 codon of ApoE gene
cgcggacatggaggacgtg

SEQ ID NO: 27 - DNA, 20 bp, Artificial Sequence
  X part of Single nucleic acid for detecting SNP in 112 codon of ApoE gene
gcgcggacatggaggacgtg

SEQ ID NO: 28 - DNA, 21 bp, Artificial Sequence
  X part of Single nucleic acid for detecting SNP in 112 codon of ApoE gene
ggcgcggacatggaggacgtg

SEQ ID NO: 29 - DNA, 22 bp, Artificial Sequence
  X part of Single nucleic acid for detecting SNP in 112 codon of ApoE gene
gggcgcggacatggaggacgtg

SEQ ID NO: 30 - DNA, 23 bp, Artificial Sequence
  X part of Single nucleic acid for detecting SNP in 112 codon of ApoE gene
tgggcgcggacatggaggacgtg

SEQ ID NO: 31 - DNA, 24 bp, Artificial Sequence
  X part of Single nucleic acid for detecting SNP in 112 codon of ApoE gene
ctgggcgcggacatggaggacgtg

SEQ ID NO: 32 - DNA, 25 bp, Artificial Sequence
  X part of Single nucleic acid for detecting SNP in 112 codon of ApoE gene
gctgggcgcggacatggaggacgtg

SEQ ID NO: 33 - DNA, 26 bp, Artificial Sequence
  X part of Single nucleic acid for detecting SNP in 112 codon of ApoE gene
ggctgggcgcggacatggaggacgtg

SEQ ID NO: 34 - DNA, 27 bp, Artificial Sequence
  X part of Single nucleic acid for detecting SNP in 112 codon of ApoE gene
cggctgggcgcggacatggaggacgtg

SEQ ID NO: 35 - DNA, 28 bp, Artificial Sequence
  X part of Single nucleic acid for detecting SNP in 112 codon of ApoE gene
ccggctgggcgcggacatggaggacgtg

SEQ ID NO: 36 - DNA, 29 bp, Artificial Sequence
  X part of Single nucleic acid for detecting SNP in 112 codon of ApoE gene
cccggctgggcgcggacatggaggacgtg

SEQ ID NO: 37 - DNA, 30 bp, Artificial Sequence
  X part of Single nucleic acid for detecting SNP in 112 codon of ApoE gene
gcccggctgggcgcggacatggaggacgtg

SEQ ID NO: 38 - DNA, 4 bp, Artificial Sequence
  X part of Single nucleic acid for detecting SNP in 152 codon of ApoE gene
gaag

SEQ ID NO: 39 - DNA, 5 bp, Artificial Sequence
  X part of Single nucleic acid for detecting SNP in 152 codon of ApoE gene
agaag

SEQ ID NO: 40 - DNA, 6 bp, Artificial Sequence
  X part of Single nucleic acid for detecting SNP in 152 codon of ApoE gene
cagaag

SEQ ID NO: 41 - DNA, 7 bp, Artificial Sequence
  X part of Single nucleic acid for detecting SNP in 152 codon of ApoE gene
gcagaag

SEQ ID NO: 42 - DNA, 8 bp, Artificial Sequence
  X part of Single nucleic acid for detecting SNP in 152 codon of ApoE gene
tgcagaag

SEQ ID NO: 43 - DNA, 9 bp, Artificial Sequence
  X part of Single nucleic acid for detecting SNP in 152 codon of ApoE gene
ctgcagaag

SEQ ID NO: 44 - DNA, 10 bp, Artificial Sequence
  X part of Single nucleic acid for detecting SNP in 152 codon of ApoE gene
cctgcagaag

SEQ ID NO: 45 - DNA, 11 bp, Artificial Sequence
  X part of Single nucleic acid for detecting SNP in 152 codon of ApoE gene
acctgcagaag

SEQ ID NO: 46 - DNA, 12 bp, Artificial Sequence
  X part of Single nucleic acid for detecting SNP in 152 codon of ApoE gene
gacctgcagaag

SEQ ID NO: 47 - DNA, 13 bp, Artificial Sequence
  X part of Single nucleic acid for detecting SNP in 152 codon of ApoE gene
tgacctgcagaag

SEQ ID NO: 48 - DNA, 14 bp, Artificial Sequence
  X part of Single nucleic acid for detecting SNP in 152 codon of ApoE gene
atgacctgcagaag

SEQ ID NO: 49 - DNA, 15 bp, Artificial Sequence
  X part of Single nucleic acid for detecting SNP in 152 codon of ApoE gene
gatgacctgcagaag

SEQ ID NO: 50 - DNA, 16 bp, Artificial Sequence
  X part of Single nucleic acid for detecting SNP in 152 codon of ApoE gene
cgatgacctgcagaag

SEQ ID NO: 51 - DNA, 17 bp, Artificial Sequence
  X part of Single nucleic acid for detecting SNP in 152 codon of ApoE gene
ccgatgacctgcagaag

SEQ ID NO: 52 - DNA, 18 bp, Artificial Sequence
  X part of Single nucleic acid for detecting SNP in 152 codon of ApoE gene
gccgatgacctgcagaag

SEQ ID NO: 53 - DNA, 19 bp, Artificial Sequence
  X part of Single nucleic acid for detecting SNP in 152 codon of ApoE gene
tgccgatgacctgcagaag

SEQ ID NO: 54 - DNA, 20 bp, Artificial Sequence
  X part of Single nucleic acid for detecting SNP in 152 codon of ApoE gene
atgccgatgacctgcagaag

SEQ ID NO: 55 - DNA, 21 bp, Artificial Sequence
  X part of Single nucleic acid for detecting SNP in 152 codon of ApoE gene
gatgccgatgacctgcagaag

SEQ ID NO: 56 - DNA, 22 bp, Artificial Sequence
  X part of Single nucleic acid for detecting SNP in 152 codon of ApoE gene
cgatgccgatgacctgcagaag

SEQ ID NO: 57 - DNA, 23 bp, Artificial Sequence
  X part of Single nucleic acid for detecting SNP in 152 codon of ApoE gene
gcgatgccgatgacctgcagaag

SEQ ID NO: 58 - DNA, 24 bp, Artificial Sequence
  X part of Single nucleic acid for detecting SNP in 152 codon of ApoE gene
cgcgatgccgatgacctgcagaag

SEQ ID NO: 59 - DNA, 25 bp, Artificial Sequence
  X part of Single nucleic acid for detecting SNP in 152 codon of ApoE gene
ccgcgatgccgatgacctgcagaag

SEQ ID NO: 60 - DNA, 26 bp, Artificial Sequence
  X part of Single nucleic acid for detecting SNP in 152 codon of ApoE gene
tccgcgatgccgatgacctgcagaag

SEQ ID NO: 61 - DNA, 27 bp, Artificial Sequence
  X part of Single nucleic acid for detecting SNP in 152 codon of ApoE gene
ctccgcgatgccgatgacctgcagaag

SEQ ID NO: 62 - DNA, 28 bp, Artificial Sequence
  X part of Single nucleic acid for detecting SNP in 152 codon of ApoE gene
cctccgcgatgccgatgacctgcagaag

SEQ ID NO: 63 - DNA, 29 bp, Artificial Sequence
  X part of Single nucleic acid for detecting SNP in 152 codon of ApoE gene
tcctccgcgatgccgatgacctgcagaag

SEQ ID NO: 64 - DNA, 30 bp, Artificial Sequence
  X part of Single nucleic acid for detecting SNP in 152 codon of ApoE gene
ctcctccgcgatgccgatgacctgcagaag

SEQ ID NO: 65 - DNA, 1 bp, Artificial Sequence
  Z part of Single nucleic acid for detecting SNP in 112 codon of ApoE gene
g

SEQ ID NO: 66 - DNA, 2 bp, Artificial Sequence
  Z part of Single nucleic acid for detecting SNP in 112 codon of ApoE gene
gc

SEQ ID NO: 67 - DNA, 3 bp, Artificial Sequence
  Z part of Single nucleic acid for detecting SNP in 112 codon of ApoE gene
gcg

SEQ ID NO: 68 - DNA, 4 bp, Artificial Sequence
  Z part of Single nucleic acid for detecting SNP in 112 codon of ApoE gene
gcgg

SEQ ID NO: 69 - DNA, 5 bp, Artificial Sequence
  Z part of Single nucleic acid for detecting SNP in 112 codon of ApoE gene
gcggc

SEQ ID NO: 70 - DNA, 6 bp, Artificial Sequence
  Z part of Single nucleic acid for detecting SNP in 112 codon of ApoE gene
gcggcc

SEQ ID NO: 71 - DNA, 7 bp, Artificial Sequence
  Z part of Single nucleic acid for detecting SNP in 112 codon of ApoE gene
gcggccg

SEQ ID NO: 72 - DNA, 8 bp, Artificial Sequence
  Z part of Single nucleic acid for detecting SNP in 112 codon of ApoE gene
gcggccgc

SEQ ID NO: 73 - DNA, 9 bp, Artificial Sequence
  Z part of Single nucleic acid for detecting SNP in 112 codon of ApoE gene
gcggccgcc

SEQ ID NO: 74 - DNA, 10 bp, Artificial Sequence
  Z part of Single nucleic acid for detecting SNP in 112 codon of ApoE gene
gcggccgcct

SEQ ID NO: 75 - DNA, 11 bp, Artificial Sequence
  Z part of Single nucleic acid for detecting SNP in 112 codon of ApoE gene
gcggccgcctg

SEQ ID NO: 76 - DNA, 12 bp, Artificial Sequence
  Z part of Single nucleic acid for detecting SNP in 112 codon of ApoE gene
gcggccgcctgg

SEQ ID NO: 77 - DNA, 13 bp, Artificial Sequence
  Z part of Single nucleic acid for detecting SNP in 112 codon of ApoE gene
gcggccgcctggt

SEQ ID NO: 78 - DNA, 14 bp, Artificial Sequence
  Z part of Single nucleic acid for detecting SNP in 112 codon of ApoE gene
gcggccgcctggtg

SEQ ID NO: 79 - DNA, 15 bp, Artificial Sequence
  Z part of Single nucleic acid for detecting SNP in 112 codon of ApoE gene
gcggccgcctggtgc

SEQ ID NO: 80 - DNA, 16 bp, Artificial Sequence
  Z part of Single nucleic acid for detecting SNP in 112 codon of ApoE gene
gcggccgcctggtgca

SEQ ID NO: 81 - DNA, 17 bp, Artificial Sequence
  Z part of Single nucleic acid for detecting SNP in 112 codon of ApoE gene
gcggccgcctggtgcag

SEQ ID NO: 82 - DNA, 18 bp, Artificial Sequence
  Z part of Single nucleic acid for detecting SNP in 112 codon of ApoE gene
gcggccgcctggtgcagt

SEQ ID NO: 83 - DNA, 19 bp, Artificial Sequence
  Z part of Single nucleic acid for detecting SNP in 112 codon of ApoE gene
gcggccgcctggtgcagta

SEQ ID NO: 84 - DNA, 20 bp, Artificial Sequence
  Z part of Single nucleic acid for detecting SNP in 112 codon of ApoE gene
gcggccgcctggtgcagtac

SEQ ID NO: 85 - DNA, 1 bp, Artificial Sequence
  Z part of Single nucleic acid for detecting SNP in 152 codon of ApoE gene
g

SEQ ID NO: 86 - DNA, 2 bp, Artificial Sequence
  Z part of Single nucleic acid for detecting SNP in 152 codon of ApoE gene
gc

SEQ ID NO: 87 - DNA, 3 bp, Artificial Sequence
  Z part of Single nucleic acid for detecting SNP in 152 codon of ApoE gene
gcc

SEQ ID NO: 88 - DNA, 4 bp, Artificial Sequence
  Z part of Single nucleic acid for detecting SNP in 152 codon of ApoE gene
gcct

SEQ ID NO: 89 - DNA, 5 bp, Artificial Sequence
  Z part of Single nucleic acid for detecting SNP in 152 codon of ApoE gene
gcctg

SEQ ID NO: 90 - DNA, 6 bp, Artificial Sequence
  Z part of Single nucleic acid for detecting SNP in 152 codon of ApoE gene
gcctgg

SEQ ID NO: 91 - DNA, 7 bp, Artificial Sequence
  Z part of Single nucleic acid for detecting SNP in 152 codon of ApoE gene
gcctggc

SEQ ID NO: 92 - DNA, 8 bp, Artificial Sequence
  Z part of Single nucleic acid for detecting SNP in 152 codon of ApoE gene
gcctggca

SEQ ID NO: 93 - DNA, 9 bp, Artificial Sequence
  Z part of Single nucleic acid for detecting SNP in 152 codon of ApoE gene
gcctggcag

SEQ ID NO: 94 - DNA, 10 bp, Artificial Sequence
  Z part of Single nucleic acid for detecting SNP in 152 codon of ApoE gene
gcctggcagt

SEQ ID NO: 95 - DNA, 11 bp, Artificial Sequence
  Z part of Single nucleic acid for detecting SNP in 152 codon of ApoE gene
gcctggcagtg

SEQ ID NO: 96 - DNA, 12 bp, Artificial Sequence
  Z part of Single nucleic acid for detecting SNP in 152 codon of ApoE gene
gcctggcagtgt

SEQ ID NO: 97 - DNA, 13 bp, Artificial Sequence
  Z part of Single nucleic acid for detecting SNP in 152 codon of ApoE gene
gcctggcagtgta

SEQ ID NO: 98 - DNA, 14 bp, Artificial Sequence
  Z part of Single nucleic acid for detecting SNP in 152 codon of ApoE gene
gcctggcagtgtac

SEQ ID NO: 99 - DNA, 15 bp, Artificial Sequence
  Z part of Single nucleic acid for detecting SNP in 152 codon of ApoE gene
gcctggcagtgtacc

SEQ ID NO: 100 - DNA, 16 bp, Artificial Sequence
  Z part of Single nucleic acid for detecting SNP in 152 codon of ApoE gene
gcctggcagtgtacca

SEQ ID NO: 101 - DNA, 17 bp, Artificial Sequence
  Z part of Single nucleic acid for detecting SNP in 152 codon of ApoE gene
gcctggcagtgtaccag

SEQ ID NO: 102 - DNA, 18 bp, Artificial Sequence
  Z part of Single nucleic acid for detecting SNP in 152 codon of ApoE gene
gcctggcagtgtaccagg

SEQ ID NO: 103 - DNA, 19 bp, Artificial Sequence
  Z part of Single nucleic acid for detecting SNP in 152 codon of ApoE gene
gcctggcagtgtaccaggc

SEQ ID NO: 104 - DNA, 20 bp, Artificial Sequence
  Z part of Single nucleic acid for detecting SNP in 152 codon of ApoE gene
gcctggcagtgtaccaggcc